European Patent Application EP 4 464 721 A2, published November 20, 2024. Title: HETEROTANDEM BICYCLIC PEPTIDE COMPLEXES. Applicant: BicycleTX Limited. The sequence listing filed with the application follows.

SEQUENCE LISTING (84 sequences)

SEQ ID NO: 1 - protein, 20 aa, synthetic construct
  REGION 1..20: note = Synthetic Peptide
  SITE 2: note = Xaa - Homoarginine
DXCSAGWLTMCQKLHLCPSH

SEQ ID NO: 2 - protein, 20 aa, synthetic construct
  REGION 1..20: note = Synthetic Peptide
  SITE 2: note = Xaa - Homoarginine
DXCSKGWLTMCQKLHLCPSH

SEQ ID NO: 3 - protein, 20 aa, synthetic construct
  REGION 1..20: note = Synthetic Peptide
  SITE 2: note = Xaa - Homoarginine
DXCSAGWLTKCQKLHLCPSH

SEQ ID NO: 4 - protein, 20 aa, synthetic construct
  REGION 1..20: note = Synthetic Peptide
  SITE 2: note = Xaa - Homoarginine
DXCSAGWLTMCKKLHLCPSH

SEQ ID NO: 5 - protein, 20 aa, synthetic construct
  REGION 1..20: note = Synthetic Peptide
  SITE 2: note = Xaa - Homoarginine
DXCSAGWLTMCQKLKLCPSH

SEQ ID NO: 6 - protein, 21 aa, synthetic construct
  REGION 1..21: note = Synthetic Peptide
SDKCSAGWLTMCQKLHLCPSH

SEQ ID NO: 7 - protein, 22 aa, synthetic construct
  REGION 1..22: note = Synthetic Peptide
  SITE 3: note = Xaa - Homoarginine
  SITE 14: note = Xaa - Homoarginine
SDXCSAGWLTMCQXLHLCPSHK

SEQ ID NO: 8 - protein, 22 aa, synthetic construct
  REGION 1..22: note = Synthetic Peptide
  SITE 3: note = Xaa - Homoarginine
  SITE 13: note = Xaa - Homoarginine
SDXCSAGWLTMCXQLNLCPSHK

SEQ ID NO: 9 - protein, 21 aa, synthetic construct
  REGION 1..21: note = Synthetic Peptide
SDKCSAGWLTMCQKLHLCPSH

SEQ ID NO: 10 - protein, 18 aa, synthetic construct
  REGION 1..18: note = Synthetic Peptide
  SITE 2: note = Xaa - Homoarginine
  SITE 5: note = Xaa - hydroxyproline
  SITE 17: note = Xaa - Homoarginine
AXDCXLVNPLCLHPDWXC

SEQ ID NO: 11 - protein, 19 aa, synthetic construct
  REGION 1..19: note = Synthetic Peptide
  SITE 2: note = Xaa - Homoarginine
  SITE 5: note = Xaa - hydroxyproline
  SITE 17: note = Xaa - Homoarginine
AXDCXLVNPLCLHPDWXCK

SEQ ID NO: 12 - protein, 18 aa, synthetic construct
  REGION 1..18: note = Synthetic Peptide
  SITE 2: note = Xaa - Homoarginine
  SITE 5: note = Xaa - hydroxyproline
  SITE 17: note = Xaa - Homoarginine
AXDCXLVNPLCLKPDWXC

SEQ ID NO: 13 - protein, 18 aa, synthetic construct
  REGION 1..18: note = Synthetic Peptide
  SITE 2: note = Xaa - Homoarginine
  SITE 5: note = Xaa - hydroxyproline
  SITE 17: note = Xaa - Homoarginine
AXDCXKVNPLCLHPDWXC

SEQ ID NO: 14 - protein, 18 aa, synthetic construct
  REGION 1..18: note = Synthetic Peptide
  SITE 2: note = Xaa - Homoarginine
  SITE 5: note = Xaa - hydroxyproline
  SITE 17: note = Xaa - Homoarginine
AXDCXLVNPLCKHPDWXC

SEQ ID NO: 15 - protein, 18 aa, synthetic construct
  REGION 1..18: note = Synthetic Peptide
  SITE 2: note = Xaa - Homoarginine
  SITE 5: note = Xaa - hydroxyproline
  SITE 17: note = Xaa - Homoarginine
AXDCXLVNPLCLHPDWXC

SEQ ID NO: 16 - protein, 19 aa, synthetic construct
  REGION 1..19: note = Synthetic Peptide
  SITE 2: note = Xaa - Homoarginine
  SITE 5: note = Xaa - hydroxyproline
  SITE 17: note = Xaa - Homoarginine
AXDCXLVNPLCLHPDWXCK

SEQ ID NO: 17 - protein, 18 aa, synthetic construct
  REGION 1..18: note = Synthetic Peptide
  SITE 2: note = Xaa - Homoarginine
  SITE 5: note = Xaa - hydroxyproline
  SITE 17: note = Xaa - Homoarginine
AXDCXLVNPLCLKPDWXC

SEQ ID NO: 18 - protein, 18 aa, synthetic construct
  REGION 1..18: note = Synthetic Peptide
  SITE 2: note = Xaa - Homoarginine
  SITE 5: note = Xaa - hydroxyproline
  SITE 17: note = Xaa - Homoarginine
AXDCXKVNPLCLHPDWXC

SEQ ID NO: 19 - protein, 18 aa, synthetic construct
  REGION 1..18: note = Synthetic Peptide
  SITE 2: note = Xaa - Homoarginine
  SITE 5: note = Xaa - hydroxyproline
  SITE 17: note = Xaa - Homoarginine
AXDCXLVNPLCKHPDWXC

SEQ ID NO: 20 - protein, 18 aa, synthetic construct
  REGION 1..18: note = Synthetic Peptide
  SITE 2: note = Xaa - Homoarginine
  SITE 5: note = Xaa - hydroxyproline
  SITE 17: note = Xaa - Homoarginine
AXDCXLVNPLCLHPEWXC

SEQ ID NO: 21 - protein, 18 aa, synthetic construct
  REGION 1..18: note = Synthetic Peptide
  SITE 2: note = Xaa - Homoarginine
  SITE 5: note = Xaa - hydroxyproline
  SITE 17: note = Xaa - Homoarginine
AXECXLVNPLCLHPEWXC

SEQ ID NO: 22 - protein, 18 aa, synthetic construct
  REGION 1..18: note = Synthetic Peptide
  SITE 2: note = Xaa - Homoarginine
  SITE 5: note = Xaa - hydroxyproline
  SITE 17: note = Xaa - Homoarginine
AXDCXLVNPLCLEPDWXC

SEQ ID NO: 23 - protein, 18 aa, synthetic construct
  REGION 1..18: note = Synthetic Peptide
  SITE 2: note = Xaa - Homoarginine
  SITE 5: note = Xaa - hydroxyproline
AXDCXLVNPLCLHPDWTC

SEQ ID NO: 24 - protein, 18 aa, synthetic construct
  REGION 1..18: note = Synthetic Peptide
  SITE 2: note = Xaa - Homoarginine
  SITE 5: note = Xaa - hydroxyproline
AXDCXLVNPLCLEPDWTC

SEQ ID NO: 25 - protein, 19 aa, synthetic construct
  REGION 1..19: note = Synthetic Peptide
  SITE 2: note = Xaa - Homoarginine
  SITE 5: note = Xaa - hydroxyproline
AXDCXLVNPLCLEPDWTCA

SEQ ID NO: 26 - protein, 18 aa, synthetic construct
  REGION 1..18: note = Synthetic Peptide
  SITE 2: note = Xaa - Homoarginine
  SITE 5: note = Xaa - hydroxyproline
AXDCXLVNPLCLEPAWTC

SEQ ID NO: 27 - protein, 18 aa, synthetic construct
  REGION 1..18: note = Synthetic Peptide
  SITE 2: note = Xaa - Homoarginine
  SITE 5: note = Xaa - hydroxyproline
  SITE 13: note = Xaa - 3,3-diphenylalanine
AXDCXLVNPLCLXPDWTC

SEQ ID NO: 28 - protein, 15 aa, synthetic construct
  REGION 1..15: note = Synthetic Peptide
  SITE 2: note = Xaa - hydroxyproline
  SITE 10: note = Xaa - 3,3-diphenylalanine
CXLVNPLCLXPDWTC

SEQ ID NO: 29 - protein, 16 aa, synthetic construct
  REGION 1..16: note = Synthetic Peptide
  SITE 2: note = Xaa - hydroxyproline
CXLVNPLCLEPDWTCA

SEQ ID NO: 30 - protein, 18 aa, synthetic construct
  REGION 1..18: note = Synthetic Peptide
  SITE 2: note = Xaa - Homoarginine
  SITE 5: note = Xaa - hydroxyproline
  SITE 6: note = Xaa - beta-cyclobutylalanine
  SITE 17: note = Xaa - Homoarginine
AXDCXXVNPLCLHPDWXC

SEQ ID NO: 31 - protein, 18 aa, synthetic construct
  REGION 1..18: note = Synthetic Peptide
  SITE 2: note = Xaa - Homoarginine
  SITE 5: note = Xaa - hydroxyproline
  SITE 6: note = Xaa - beta-cyclobutylalanine
AXDCXXVNPLCLEPDWTC

SEQ ID NO: 32 - protein, 19 aa, synthetic construct
  REGION 1..19: note = Synthetic Peptide
  SITE 2: note = Xaa - Homoarginine
  SITE 5: note = Xaa - hydroxyproline
  SITE 6: note = Xaa - beta-cyclobutylalanine
AXDCXXVNPLCLEPDWTCA

SEQ ID NO: 33 - protein, 16 aa, synthetic construct
  REGION 1..16: note = Synthetic Peptide
  SITE 2: note = Xaa - hydroxyproline
  SITE 3: note = Xaa - beta-cyclobutylalanine
  SITE 10: note = Xaa - 3,3-diphenylalanine
CXXVNPLCLXPDWTCA

SEQ ID NO: 34 - protein, 18 aa, synthetic construct
  REGION 1..18: note = Synthetic Peptide
  SITE 2: note = Xaa - Homoarginine
  SITE 5: note = Xaa - hydroxyproline
  SITE 13: note = Xaa - 3,3-diphenylalanine
  SITE 17: note = Xaa - Homoarginine
AXDCXLVNPLCLXPDWXC

SEQ ID NO: 35 - protein, 18 aa, synthetic construct
  REGION 1..18: note = Synthetic Peptide
  SITE 2: note = Xaa - Homoarginine
  SITE 5: note = Xaa - hydroxyproline
  SITE 15: note = Xaa - D-1-naphthylalanine
  SITE 17: note = Xaa - Homoarginine
AXDCXLVNPLCLHPXWXC

SEQ ID NO: 36 - protein, 18 aa, synthetic construct
  REGION 1..18: note = Synthetic Peptide
  SITE 2: note = Xaa - Homoarginine
  SITE 5: note = Xaa - hydroxyproline
  SITE 13: note = Xaa - D-1-naphthylalanine
  SITE 17: note = Xaa - Homoarginine
AXDCXLVNPLCLXPDWXC

SEQ ID NO: 37 - protein, 18 aa, synthetic construct
  REGION 1..18: note = Synthetic Peptide
  SITE 2: note = Xaa - Homoarginine
  SITE 5: note = Xaa - hydroxyproline
  SITE 15: note = Xaa - D-1-naphthylalanine
AXDCXLVNPLCLEPXWTC

SEQ ID NO: 38 - protein, 15 aa, synthetic construct
  REGION 1..15: note = Synthetic Peptide
  SITE 2: note = Xaa - hydroxyproline
  SITE 10: note = Xaa - 1-naphthylalanine
CXLVNPLCLXPDWTC

SEQ ID NO: 39 - protein, 16 aa, synthetic construct
  REGION 1..16: note = Synthetic Peptide
  SITE 2: note = Xaa - hydroxyproline
  SITE 10: note = Xaa - 3,3-diphenylalanine
CXLVNPLCLXPDWTCK

SEQ ID NO: 40 - protein, 18 aa, synthetic construct
  REGION 1..18: note = Synthetic Peptide
  SITE 1: note = Xaa - N-methyl-alanine
  SITE 2: note = Xaa - Homoarginine
  SITE 5: note = Xaa - hydroxyproline
  SITE 17: note = Xaa - Homoarginine
XXDCXLVNPLCLHPDWXC

SEQ ID NO: 41 - protein, 18 aa, synthetic construct
  REGION 1..18: note = Synthetic Peptide
  SITE 1: note = Xaa - N-methyl-alanine
  SITE 2: note = Xaa - Homoarginine
  SITE 5: note = Xaa - hydroxyproline
XXDCXLVNPLCLEPDWTC

SEQ ID NO: 42 - protein, 19 aa, synthetic construct
  REGION 1..19: note = Synthetic Peptide
  SITE 2: note = Xaa - Homoarginine
  SITE 5: note = Xaa - hydroxyproline
  SITE 6: note = Xaa - beta-cyclobutylalanine
AXDCXXVNPLCLEPAWTCA

SEQ ID NO: 43 - protein, 19 aa, synthetic construct
  REGION 1..19: note = Synthetic Peptide
  SITE 1: note = Xaa - D-1-naphthylalanine
  SITE 2: note = Xaa - Homoarginine
  SITE 5: note = Xaa - hydroxyproline
  SITE 6: note = Xaa - beta-cyclobutylalanine
XXDCXXVNPLCLEPAWTCA

SEQ ID NO: 44 - protein, 18 aa, synthetic construct
  REGION 1..18: note = Synthetic Peptide
  SITE 5: note = Xaa - hydroxyproline
AEDCXLVNPLCLEPDWTC

SEQ ID NO: 45 - protein, 18 aa, synthetic construct
  REGION 1..18: note = Synthetic Peptide
  SITE 5: note = Xaa - hydroxyproline
AADCXLVNPLCLEPDWTC

SEQ ID NO: 46 - protein, 17 aa, synthetic construct
  REGION 1..17: note = Synthetic Peptide
  SITE 4: note = Xaa - hydroxyproline
ADCXLVNPLCLEPDWTC

SEQ ID NO: 47 - protein, 18 aa, synthetic construct
  REGION 1..18: note = Synthetic Peptide
  SITE 2: note = Xaa - Homoarginine
  SITE 5: note = Xaa - hydroxyproline
  SITE 6: note = Xaa - homoglutamic acid
  SITE 17: note = Xaa - Homoarginine
AXDCXXVNPLCLHPDWXC

SEQ ID NO: 48 - protein, 18 aa, synthetic construct
  REGION 1..18: note = Synthetic Peptide
  SITE 2: note = Xaa - Homoarginine
  SITE 5: note = Xaa - hydroxyproline
  SITE 12: note = Xaa - homoglutamic acid
  SITE 17: note = Xaa - Homoarginine
AXDCXLVNPLCXHPDWXC

SEQ ID NO: 49 - protein, 18 aa, synthetic construct
  REGION 1..18: note = Synthetic Peptide
  SITE 2: note = Xaa - Homoarginine
  SITE 5: note = Xaa - hydroxyproline
  SITE 13: note = Xaa - homoglutamic acid
  SITE 17: note = Xaa - Homoarginine
AXDCXLVNPLCLXPDWXC

SEQ ID NO: 50 - protein, 18 aa, synthetic construct
  REGION 1..18: note = Synthetic Peptide
  SITE 2: note = Xaa - Homoarginine
  SITE 5: note = Xaa - hydroxyproline
  SITE 15: note = Xaa - D-norleucine
  SITE 17: note = Xaa - Homoarginine
AXDCXLVNPLCLHPXWXC

SEQ ID NO: 51 - protein, 18 aa, synthetic construct
  REGION 1..18: note = Synthetic Peptide
  SITE 2: note = Xaa - Homoarginine
  SITE 5: note = Xaa - hydroxyproline
  SITE 13: note = Xaa - X is Nle
  SITE 17: note = Xaa - Homoarginine
AXDCXLVNPLCLXPDWXC

SEQ ID NO: 52 - protein, 15 aa, synthetic construct
  REGION 1..15: note = Synthetic Peptide
  SITE 3: note = Xaa - 1-naphthylalanine
  SITE 7: note = Xaa - Homoarginine
  SITE 13: note = Xaa - hydroxyproline
CPXDCMXDWSTPXWC

SEQ ID NO: 53 - protein, 15 aa, synthetic construct
  REGION 1..15: note = Synthetic Peptide
  SITE 3: note = Xaa - 1-naphthylalanine
  SITE 7: note = Xaa - Homoarginine
  SITE 13: note = Xaa - hydroxyproline
CPXKCMXDWSTPXWC

SEQ ID NO: 54 - protein, 15 aa, synthetic construct
  REGION 1..15: note = Synthetic Peptide
  SITE 1: note = Xaa - 3-mercaptopropionic acid
  SITE 3: note = Xaa - 1-naphthylalanine
  SITE 7: note = Xaa - Homoarginine
  SITE 13: note = Xaa - hydroxyproline
XPXKCMXDWSTPXWC

SEQ ID NO: 55 - protein, 15 aa, synthetic construct
  REGION 1..15: note = Synthetic Peptide
  SITE 3: note = Xaa - 1-naphthylalanine
  SITE 7: note = Xaa - Homoarginine
  SITE 13: note = Xaa - hydroxyproline
  SITE 15: note = Xaa - Cysteamine
CPXKCMXDWSTPXWX

SEQ ID NO: 56 - protein, 15 aa, synthetic construct
  REGION 1..15: note = Synthetic Peptide
  SITE 1: note = Xaa - 3-mercaptopropionic acid
  SITE 3: note = Xaa - 1-naphthylalanine
  SITE 7: note = Xaa - Homoarginine
  SITE 13: note = Xaa - hydroxyproline
  SITE 15: note = Xaa - Cysteamine
XPXKCMXDWSTPXWX

SEQ ID NO: 57 - protein, 15 aa, synthetic construct
  REGION 1..15: note = Synthetic Peptide
  SITE 3: note = Xaa - 1-naphthylalanine
  SITE 7: note = Xaa - Homoarginine
  SITE 13: note = Xaa - hydroxyproline
CPXKCMXHWSTPXWC

SEQ ID NO: 58 - protein, 15 aa, synthetic construct
  REGION 1..15: note = Synthetic Peptide
  SITE 3: note = Xaa - 1-naphthylalanine
  SITE 7: note = Xaa - Homoarginine
  SITE 13: note = Xaa - hydroxyproline
CPXKCMXEWSTPXWC

SEQ ID NO: 59 - protein, 15 aa, synthetic construct
  REGION 1..15: note = Synthetic Peptide
  SITE 3: note = Xaa - 1-naphthylalanine
  SITE 7: note = Xaa - Homoarginine
  SITE 13: note = Xaa - hydroxyproline
CPXECMXDWSTPXWC

SEQ ID NO: 60 - protein, 15 aa, synthetic construct
  REGION 1..15: note = Synthetic Peptide
  SITE 3: note = Xaa - 1-naphthylalanine
  SITE 7: note = Xaa - Homoarginine
  SITE 13: note = Xaa - hydroxyproline
CPXACMXDWSTPXWC

SEQ ID NO: 61 - protein, 15 aa, synthetic construct
  REGION 1..15: note = Synthetic Peptide
  SITE 3: note = Xaa - 1-naphthylalanine
  SITE 7: note = Xaa - Homoarginine
  SITE 13: note = Xaa - hydroxyproline
CPXECLXDWSTPXWC

SEQ ID NO: 62 - protein, 18 aa, synthetic construct
  REGION 1..18: note = Synthetic Peptide
  SITE 1: note = Xaa - palmitic acid
  REGION 2..3: note = Xaa - X is yGlu
  SITE 6: note = Xaa - 1-naphthylalanine
  SITE 10: note = Xaa - Homoarginine
  SITE 16: note = Xaa - hydroxyproline
XXXCPXKCMXDWSTPXWC

SEQ ID NO: 63 - protein, 15 aa, synthetic construct
  REGION 1..15: note = Synthetic Peptide
  SITE 3: note = Xaa - 1-naphthylalanine
  SITE 7: note = Xaa - Homoarginine
  SITE 13: note = Xaa - hydroxyproline
CPXECMXEWSTPXWC

SEQ ID NO: 64 - protein, 17 aa, synthetic construct
  REGION 1..17: note = Synthetic Peptide
  SITE 1: note = Xaa - 4-pentynoic acid
  SITE 2: note = Xaa - beta-alanine
  SITE 5: note = Xaa - 1-naphthylalanine
  SITE 9: note = Xaa - Homoarginine
  SITE 15: note = Xaa - hydroxyproline
XXCPXDCMXDWSTPXWC

SEQ ID NO: 65 - protein, 17 aa, synthetic construct
  REGION 1..17: note = Synthetic Peptide
  SITE 1: note = Xaa - 4-pentynoic acid
  SITE 2: note = Xaa - beta-alanine
  SITE 5: note = Xaa - 1-naphthylalanine
  SITE 9: note = Xaa - Homoarginine
  SITE 15: note = Xaa - hydroxyproline
XXCPXKCMXDWSTPXWC

SEQ ID NO: 66 - protein, 16 aa, synthetic construct
  REGION 1..16: note = Synthetic Peptide
  SITE 1: note = Xaa - 4-pentynoic acid
  SITE 4: note = Xaa - 1-naphthylalanine
  SITE 8: note = Xaa - Homoarginine
  SITE 14: note = Xaa - hydroxyproline
XCPXDCMXDWSTPXWC

SEQ ID NO: 67 - protein, 16 aa, synthetic construct
  REGION 1..16: note = Synthetic Peptide
  SITE 2: note = Xaa - t-butyl-alanine
  SITE 5: note = Xaa - D-lysine(4-pentynoic acid)
  SITE 14: note = Xaa - X is Nle
CXPEXPYCFADPYXCA

SEQ ID NO: 68 - protein, 16 aa, synthetic construct
  REGION 1..16: note = Synthetic Peptide
  SITE 2: note = Xaa - t-butyl-alanine
  SITE 14: note = Xaa - X is Nle
  SITE 16: note = Xaa - diaminopropionic acid (4-pentynoic acid)
CXEEKPYCFADPYXCX

SEQ ID NO: 69 - protein, 16 aa, synthetic construct
  REGION 1..16: note = Synthetic Peptide
  SITE 2: note = Xaa - t-butyl-alanine
  SITE 14: note = Xaa - X is Nle
  SITE 16: note = Xaa - diaminopropionic acid (4-pentynoic acid)
CXPEKPYCFADPYXCX

SEQ ID NO: 70 - protein, 16 aa, synthetic construct
  REGION 1..16: note = Synthetic Peptide
  SITE 2: note = Xaa - t-butyl-alanine
  SITE 14: note = Xaa - X is Nle
CXPEKPYCFADPYXCA

SEQ ID NO: 71 - protein, 15 aa, synthetic construct
  REGION 1..15: note = Synthetic Peptide
  SITE 2: note = Xaa - t-butyl-alanine
  SITE 14: note = Xaa - X is Nle
CXEEKPYCFADPYXC

SEQ ID NO: 72 - protein, 15 aa, synthetic construct
  REGION 1..15: note = Synthetic Peptide
  SITE 2: note = Xaa - t-butyl-alanine
  SITE 14: note = Xaa - X is Nle
CXPEKPYCFADPYXC

SEQ ID NO: 73 - protein, 15 aa, synthetic construct
  REGION 1..15: note = Synthetic Peptide
  SITE 2: note = Xaa - t-butyl-alanine
  SITE 14: note = Xaa - X is Nle
CXPEKPYCFANPYXC

SEQ ID NO: 74 - protein, 15 aa, synthetic construct
  REGION 1..15: note = Synthetic Peptide
  SITE 2: note = Xaa - t-butyl-alanine
  SITE 14: note = Xaa - X is Nle
CXPEKPYCFAEPYXC

SEQ ID NO: 75 - protein, 15 aa, synthetic construct
  REGION 1..15: note = Synthetic Peptide
  SITE 2: note = Xaa - t-butyl-alanine
  SITE 11: note = Xaa - X is Aad
  SITE 14: note = Xaa - X is Nle
CXPEKPYCFAXPYXC

SEQ ID NO: 76 - protein, 15 aa, synthetic construct
  REGION 1..15: note = Synthetic Peptide
  SITE 2: note = Xaa - t-butyl-alanine
  SITE 14: note = Xaa - X is Nle
  SITE 15: note = Xaa - Cysteamine
CXPEKPYCFADPYXX

SEQ ID NO: 77 - protein, 15 aa, synthetic construct
  REGION 1..15: note = Synthetic Peptide
  SITE 1: note = Xaa - 3-mercaptopropionic acid
  SITE 2: note = Xaa - t-butyl-alanine
  SITE 14: note = Xaa - X is Nle
XXPEKPYCFADPYXC

SEQ ID NO: 78 - protein, 15 aa, synthetic construct
  REGION 1..15: note = Synthetic Peptide
  SITE 1: note = Xaa - 3-mercaptopropionic acid
  SITE 2: note = Xaa - t-butyl-alanine
  SITE 14: note = Xaa - X is Nle
  SITE 15: note = Xaa - Cysteamine
XXPEKPYCFADPYXX

SEQ ID NO: 79 - protein, 18 aa, synthetic construct
  REGION 1..18: note = Synthetic Peptide
  SITE 1: note = Xaa - Palmitic acid
  REGION 2..3: note = Xaa - X is yGlu
  SITE 5: note = Xaa - t-butyl-alanine
  SITE 17: note = Xaa - X is Nle
XXXCXPEKPYCFADPYXC

SEQ ID NO: 80 - protein, 15 aa, synthetic construct
  REGION 1..15: note = Synthetic Peptide
  SITE 1: note = Xaa - 3-mercaptopropionic acid
  SITE 2: note = Xaa - t-butyl-alanine
  SITE 14: note = Xaa - X is Nle
XXEEKPYCFADPYXC

SEQ ID NO: 81 - protein, 17 aa, synthetic construct
  REGION 1..17: note = Synthetic Peptide
  SITE 15: note = Xaa - X is Nle
ACIEEKQYCFADPYXCA

SEQ ID NO: 82 - protein, 15 aa, synthetic construct
  REGION 1..15: note = Synthetic Peptide
  SITE 2: note = Xaa - t-butyl-alanine
  SITE 12: note = Xaa - N-methyl-alanine
  SITE 14: note = Xaa - X is Nle
CXPEKPYCFADXYXC

SEQ ID NO: 83 - protein, 15 aa, synthetic construct
  REGION 1..15: note = Synthetic Peptide
  SITE 2: note = Xaa - t-butyl-alanine
  SITE 12: note = Xaa - N-methyl-D-alanine
  SITE 14: note = Xaa - X is Nle
CXPEKPYCFADXYXC

SEQ ID NO: 84 - protein, 16 aa, synthetic construct
  REGION 1..16: note = Synthetic Peptide
  SITE 2: note = Xaa - t-butyl-alanine
  SITE 14: note = Xaa - X is Nle
  SITE 16: note = Xaa - 1,2-diaminoethane
CXPEKPYCFADPYXCX